European Patent Application EP 4 470 553 A2, published December 4, 2024. Title: NOVEL THYROID PEROXIDASE AUTOANTIBODY IMMUNOASSAY. Applicant: Siemens Healthcare Diagnostics Inc. Application WO PCT/US2019/040161, filed July 1, 2019. The sequence listing filed with the application follows.

SEQUENCE LISTING (1 sequence)

SEQ ID NO: 1 - protein, 840 aa, Macaca fascicularis
ADPGYLLECTEAFFPFISRGKELLWGKPEESRVAGILEESKRLVDTAMYATMQRNLKKREILSPHQLLSFSKLPEPTSGEIARAAEIMETSIQAMKRKVNLKIQQSQHPTDALSEDLLSIIANMSGCLPYMLPPKCPNTCLANKYRPITGACNNRDHPRWGASNTALARWLPPVYEDGFSQPRGWNPSILHNGFPLPPVREVTRHVIQVSNEVVTDDDRYSDLLMAWGQYIDHDIAFTPQSTSKAAFRGGADCQVTCENQNPCFPIQLPEEARPAAGTACLPFYRSSAACGTGDQGALFGNLSTANPRQQMNGLTSFLDASTVYGSSPALERQLRNWTSAEGLLRVHARLRDSGRAYLPFAPPRAPAACAPEPGIPGETRGPCFLAGDGRASEVPSLTALHTLWLREHNRLAAALKALNAHWSADAVYQEARKVVGALHQIITLRDYVPRILGPEAFQQYVGPYEGYDSAANPTVSNVFSTAAFRFGHATIHPLVRRLDAGFQEHPGLPGLWLHETFFSPWTLLHGGGLDPLIRGLLARPAKLQVQDQLMNEELTERLFVLSNSSTLDLASINLQRGRDHGLPGYNEWREFCGLPRLETPADLSTAIASRSVADKILDLYKHPDNIDVWLGGLAENFLPRARTGPLFACLIGKQMKALRDGDWFWWENSHVFTDAQRHELEKHSLSRVICDNTGLTRVPVDAFRVGKFPEDFESCDSIPGMNLEAWRETFPQDDKCGFPESVENGDFVHCEESGRRVLVYSCRHGYELQGHEQLTCTQEGWDFQPPLCKDVNECADGAHPPCHASARCRNTKGGFQCLCADPYELGDDGRTCVDSGRLPR